European Patent Application EP 4 166 673 A1, published April 19, 2023. Title: A Fermentation Process. Applicant: LanzaTech NZ, Inc. Application EP, filed September 22, 2014. The sequence listing filed with the application follows.

SEQUENCE LISTING (2 sequences)

SEQ ID NO: 1 - DNA, 996 bp, Clostridium autoethanogenum
  source 1..996: mol_type = genomic DNA
atgagtagtattgaaaaggtttatcatgatgaagatgttaatatggatgcacttaaaggtaaggttgtagcaataatgggatatggaagtcagggaagaggacaatccaattgcctaagagacaatggagtaaatgttataattggtgcaggaaataaggatagatatccggattgggaaaatgcggaaaaagatggatttactgtatatccttttgatgaggcagttaaaaaagctgatgtagtaatgatattacttcaagaccctgctcaacctgcagtttattatgaatcaattcatcaaaatttaagaccaaatcagacactttgctttgcacatgggtttgcaatattgtatggaacaattgtgccaccagaatttgtagatgtagtactttttgttcctaatggaccaggtcctgttgtaaggcaaaaatttctagatggttcaggaatatatggtgcagttgctgtagaccaggatgttactggacatgctaaagaaacagctcttgcgattgctaaaggtgttggcagcacaagaactggtacagtatatatttcattccaacatgagactgaaggagataactttgaagaacaggttctttatggtggaacaatcaatcttatgagggcagtgtatgaaactatggctaagaatggatatccaaaatcctttgcttatgcaaaggctataaggtccattaggtcagtaattgacgatatagatcgagttggaatagaagaatatttgtcgaaaagatgcagcagaacttgtgaatttgcagttagaacttctggacccagagttattaattatgatgaaattgaaaaaatatttagagaaactgaaaaaggtgaatttgcaaaaagatggttattggaattccaatgcggtatgcctactttaaacagattgagaagaactcataagaattcgaatatggaagttgtaggaaaagagtggagagaaaagttcagtaaagaagtataa

SEQ ID NO: 2 - DNA, 1671 bp, Clostridium autoethanogenum
  source 1..1671: mol_type = genomic DNA
atgaatagagatataaaaaaagaagtccaactaaatacagctcaaatgctagtaaaatgtttagaagccgaaggagtaaagtacatctttggtattcctggtgaagaaaacctagaaataatgaatgcaatttcagattcaactattgaatttatcacaacccgtcatgagcaaggtgctgcatttatggccgacgtttatggacgtttaacaggaaaagcaggtgtttgcctatcaacactaggaccaggtgccactaacttagtaactggtgtagcagatgctgatagtgatggtgctccggttgttgctattacaggtcaagtaggtactgaaagaatgcatataacatcgcaccaatttttagacctttgcaaaatgttcgaaccaatcacaaagagaagtaaacaaatcgttcgtcctgatactgtaagtgagattataagacttgtttttaagtatgctgaaagtgaaaagcctggagcatgccacattgatttacctgtaaatattgcaaaaatgcccgtaggtgctttagaaaagcctttggaaaagaagattccaccaaaggaacatgcagatttatcaacaattgaggaagctgcaagtgaaatcttcaaagcaaaaaatcctattatcttagctggaagcggtgctataagaggaaattcttcaaaagctgttacggaatttgcaactaaattgaaaattccagtaattaatacgatgatggcaaaaggtattattccaatggataacaagtattcaatgtggacaataggtattccacaaaaagattatgtaaataaaattattgaagaggctgatttagtaattacaattggatatgatattgtagaatatgccccatccaaatggaatataaatggggacattaaaattgtgcatatcgatgcaagaccatcacacatcaataaactttatcagcccatagtagaagtagttggtgatatttcagatgctctatacaatatattgagaagaacttctagcaaagatgaaccagtaaaagctttggaaattaaatcagaaatgctagctgaacatgaaagctatgcaaatgacaatgcttttccaatgaaaccccaaagaattttaaatgatgttagaaaggtcatgggaccacatgacattgtcatatcagatgtaggtgcccataaaatgtggattgccagacattataactgctatgagcccaatacatgtattatttcaaacggttttgctacaatgggtattggtgttccaggtgcaattgcagccaaattaattaatccagataaaaaagtattggctattgttggtgatggcggtttcatgatgaataatcaagaattagaaacagccctacgtattaaaactccaattgtagttttaatatttaatgacagtaactacggtttaataaagtggaaacaagaagaacactatggtaaaagctgttatgtagattttactaatccagactttgtaaagcttgcagaaagtatgtatgcaaaaggatatcgagtagaaaaagcagaagatttaattccaactttagaagaagctttcaaacaaaatgtacctgcagttattgattgtcaagttgactatggtgaaaatataaagcttacaaagcatttaaaagaagtttatgaaaatatgtaa